European Patent Application EP 4 279 501 A2, published November 22, 2023. Title: TUMOR ENVIRONMENT-SPECIFIC EXPRESSION OF CHIMERIC ANTIGEN RECEPTORS. Applicant: THE NATIONAL INSTITUTE FOR BIOTECHNOLOGY IN THE NEGEV LTD. Application EP WO2019/159173, filed February 14, 2019. The sequence listing filed with the application follows.

SEQUENCE LISTING (47 sequences)

SEQ ID NO: 1 - skipped

SEQ ID NO: 2 - DNA, 10 bp, Homo sapiens
  source 1..10: mol_type = other DNA
gggaatttcc

SEQ ID NO: 3 - DNA, 31 bp, Homo sapiens
  source 1..31: mol_type = other DNA
gaccttgagtacgtgcgtctctgcacgtatg

SEQ ID NO: 4 - DNA, 26 bp, Homo sapiens
  source 1..26: mol_type = other DNA
gcgcttcctgacagtgacgcgagccg

SEQ ID NO: 5 - DNA, 126 bp, synthetic construct
  misc_feature 1..126: note = SYNTHETIC PROMOTER
  source 1..126: mol_type = other DNA
gggaatttccggggactttccgggaatttccggggactttccgggaatttccagagcatattaaggtgacgcgtgtggcctcgaacaccgagcgaccctgcagcgacccgcttaaaagcggccgcc

SEQ ID NO: 6 - DNA, 163 bp, synthetic construct
  misc_feature 1..163: note = SYNTHETIC PROMOTER
  source 1..163: mol_type = other DNA
ttccgggaaagggtgggcaagtttccgggaaagcagtaggtacagccttccgggaaagggtgggcaagtttccgggaaagcagtaggtttttcgcatattaaggtgacgcgtgtggcctcgaacaccgagcgaccctgcagcgacccgcttaaaaggcgcgcc

SEQ ID NO: 7 - DNA, 257 bp, synthetic construct
  misc_feature 1..257: note = SYNTHETIC PROMOTER
  source 1..257: mol_type = other DNA
ttccgggaaagggtgggcaagtttccgggaaagcagtaggtacagccttccgggaaagggtgggcaagtttccgggaaagcagtaggtacagccttccgggaaagggtgggcaagtttccgggaaagcagtaggtacagccttccgggaaagggtgggcaagtttccgggaaagcagtaggtttttcgcatattaaggtgacgcgtgtggcctcgaacaccgagcgaccctgcagcgacccgcttaaaaggcgcgcc

SEQ ID NO: 8 - DNA, 351 bp, synthetic construct
  misc_feature 1..351: note = SYNTHETIC PROMOTER
  source 1..351: mol_type = other DNA
ttccgggaaagggtgggcaagtttccgggaaagcagtaggtacagccttccgggaaagggtgggcaagtttccgggaaagcagtaggtacagccttccgggaaagggtgggcaagtttccgggaaagcagtaggtacagccttccgggaaagggtgggcaagtttccgggaaagcagtaggtacagccttccgggaaagggtgggcaagtttccgggaaagcagtaggtacagccttccgggaaagggtgggcaagtttccgggaaagcagtaggtttttcgcatattaaggtgacgcgtgtggcctcgaacaccgagcgaccctgcagcgacccgcttaaaaggcgcgcc

SEQ ID NO: 9 - DNA, 160 bp, synthetic construct
  misc_feature 1..160: note = SYNTHETIC PROMOTER
  source 1..160: mol_type = other DNA
ttccgggaaagggtgggcaagtttccgggaacccgggaatttccggggactttccgggaatttccggggactttccgggaatttccagagcatattaaggtgacgcgtgtggcctcgaacaccgagcgaccctgcagcgacccgcttaaaagcggccgcc

SEQ ID NO: 10 - DNA, 139 bp, synthetic construct
  misc_feature 1..139: note = SYNTHETIC PROMOTER
  source 1..139: mol_type = other DNA
ttccgggaaagggtgggcaagtttccgggaacccgggaatttccggggactttccgggaatttccagagcatattaaggtgacgcgtgtggcctcgaacaccgagcgaccctgcagcgacccgcttaaaagcggccgcc

SEQ ID NO: 11 - DNA, 267 bp, synthetic construct
  misc_feature 1..267: note = SYNTHETIC PROMOTER
  source 1..267: mol_type = other DNA
ttccgggaaagggtgggcaagtttccgggaaagcagtaggtacagccttccgggaaagggtgggcaagtttccgggaaagagcagggaatttccggggactttccgggaatttccggggactttccgggaatttccagagcagggaatttccggggactttccgggaatttccggggactttccgggaatttccagagcatattaaggtgacgcgtgtggcctcgaacaccgagcgaccctgcagcgacccgcttaaaaggcgcgcc

SEQ ID NO: 12 - DNA, 372 bp, synthetic construct
  misc_feature 1..372: note = SYNTHETIC PROMOTER
  source 1..372: mol_type = other DNA
ttccgggaaagggtgggcaagtttccgggaaagcagtaggtacagccttccgggaaagggtgggcaagtttccgggaaagcagtaggtacagccttccgggaaagggtgggcaagtttccgggaaagagcagggaatttccggggactttccgggaatttccggggactttccgggaatttccagagcagggaatttccggggactttccgggaatttccggggactttccgggaatttccagagcagggaatttccggggactttccgggaatttccggggactttccgggaatttccagagcatattaaggtgacgcgtgtggcctcgaacaccgagcgaccctgcagcgacccgcttaaaaggcgcgcc

SEQ ID NO: 13 - DNA, 456 bp, synthetic construct
  misc_feature 1..456: note = SYNTHETIC PROMOTER
  source 1..456: mol_type = other DNA
ttccgggaaagggtgggcaagtttccgggaaagcagtaggtacagccttccgggaaagggtgggcaagtttccgggaaagcagtaggtacagccttccgggaaagggtgggcaagtttccgggaaagcagtaggtacagccgaccttgagtacgtgcgtctctgcacgtatgagagcagaccttgagtacgtgcgtctctgcacgtatgagagcagggaatttccggggactttccgggaatttccggggactttccgggaatttccagagcagggaatttccggggactttccgggaatttccggggactttccgggaatttccagagcagggaatttccggggactttccgggaatttccggggactttccgggaatttccagagcatattaaggtgacgcgtgtggcctcgaacaccgagcgaccctgcagcgacccgcttaaaaggcgcgcc

SEQ ID NO: 14 - DNA, 446 bp, synthetic construct
  misc_feature 1..446: note = SYNTHETIC PROMOTER
  source 1..446: mol_type = other DNA
ttccgggaaagggtgggcaagtttccgggaaagcagtaggtacagccttccgggaaagggtgggcaagtttccgggaaagcagtaggtacagccttccgggaaagggtgggcaagtttccgggaaagagcagggaatttccggggactttccgggaatttccggggactttccgggaatttccagagcagggaatttccggggactttccgggaatttccggggactttccgggaatttccagagcagggaatttccggggactttccgggaatttccggggactttccgggaatttccagagcagaccttgagtacgtgcgtctctgcacgtatgagagcagaccttgagtacgtgcgtctctgcacgtatgagagcatattaaggtgacgcgtgtggcctcgaacaccgagcgaccctgcagcgacccgcttaaaaggcgcgcc

SEQ ID NO: 15 - DNA, 351 bp, synthetic construct
  misc_feature 1..351: note = SYNTHETIC PROMOTER
  source 1..351: mol_type = other DNA
ttccgggaaagggtgggcaagtttccgggaaagcagtaggtacagccttccgggaaagggtgggcaagtttccgggaaagcagtaggtacagccgaccttgagtacgtgcgtctctgcacgtatgagagcagaccttgagtacgtgcgtctctgcacgtatgagagcagggaatttccggggactttccgggaatttccggggactttccgggaatttccagagcagggaatttccggggactttccgggaatttccggggactttccgggaatttccagagcatattaaggtgacgcgtgtggcctcgaacaccgagcgaccctgcagcgacccgcttaaaaggcgcgcc

SEQ ID NO: 16 - DNA, 341 bp, synthetic construct
  misc_feature 1..341: note = SYNTHETIC PROMOTER
  source 1..341: mol_type = other DNA
ttccgggaaagggtgggcaagtttccgggaaagcagtaggtacagccttccgggaaagggtgggcaagtttccgggaaagagcagggaatttccggggactttccgggaatttccggggactttccgggaatttccagagcagggaatttccggggactttccgggaatttccggggactttccgggaatttccagagcagaccttgagtacgtgcgtctctgcacgtatgagagcagaccttgagtacgtgcgtctctgcacgtatgagagcatattaaggtgacgcgtgtggcctcgaacaccgagcgaccctgcagcgacccgcttaaaaggcgcgcc

SEQ ID NO: 17 - DNA, 341 bp, synthetic construct
  misc_feature 1..341: note = SYNTHETIC PROMOTER
  source 1..341: mol_type = other DNA
gaccttgagtacgtgcgtctctgcacgtatgagagcagaccttgagtacgtgcgtctctgcacgtatgagagcattccgggaaagggtgggcaagtttccgggaaagcagtaggtacagccttccgggaaagggtgggcaagtttccgggaaagagcagggaatttccggggactttccgggaatttccggggactttccgggaatttccagagcagggaatttccggggactttccgggaatttccggggactttccgggaatttccagagcatattaaggtgacgcgtgtggcctcgaacaccgagcgaccctgcagcgacccgcttaaaaggcgcgcc

SEQ ID NO: 18 - DNA, 246 bp, synthetic construct
  misc_feature 1..246: note = SYNTHETIC PROMOTER
  source 1..246: mol_type = other DNA
ttccgggaaagggtgggcaagtttccgggaaagcagtaggtacagccgaccttgagtacgtgcgtctctgcacgtatgagagcagaccttgagtacgtgcgtctctgcacgtatgagagcagggaatttccggggactttccgggaatttccggggactttccgggaatttccagagcatattaaggtgacgcgtgtggcctcgaacaccgagcgaccctgcagcgacccgcttaaaaggcgcgcc

SEQ ID NO: 19 - DNA, 169 bp, synthetic construct
  misc_feature 1..169: note = SYNTHETIC PROMOTER
  source 1..169: mol_type = other DNA
ttccgggaaagggtgggcaagtttccgggaacccgaccttgagtacgtgcgtctctgcacgtatgtacagcgcttcctgacagtgacgcgagccgagagcatattaaggtgacgcgtgtggcctcgaacaccgagcgaccctgcagcgacccgcttaaaagcggccgcc

SEQ ID NO: 20 - DNA, 169 bp, synthetic construct
  misc_feature 1..169: note = SYNTHETIC PROMOTER
  source 1..169: mol_type = other DNA
ttccgggaaagggtgggcaagtttccgggaacccgggaatttccggggactttccgggaatttcctacagcgcttcctgacagtgacgcgagccgagagcatattaaggtgacgcgtgtggcctcgaacaccgagcgaccctgcagcgacccgcttaaaagcggccgcc

SEQ ID NO: 21 - DNA, 174 bp, synthetic construct
  misc_feature 1..174: note = SYNTHETIC PROMOTER
  source 1..174: mol_type = other DNA
ttccgggaaagggtgggcaagtttccgggaacccgggaatttccggggactttccgggaatttcctacagaccttgagtacgtgcgtctctgcacgtatgagagcatattaaggtgacgcgtgtggcctcgaacaccgagcgaccctgcagcgacccgcttaaaagcggccgcc

SEQ ID NO: 22 - DNA, 250 bp, synthetic construct
  misc_feature 1..250: note = SYNTHETIC PROMOTER
  source 1..250: mol_type = other DNA
tacagggacagcagagatccagtttggactagcccggtcgcactagttctagaacttcccggaaatagggtgggcaagtatttccgggaaattctagagggagttcccggggactttccggggattttctctagatattaaggtgacgcgtgtggcctcgaacaccgagcgaccctgcagcgacccgcttaaaagcggccgccatgggccgccatggcctcctccgaggacgtcatcaaggagttcatgc

SEQ ID NO: 23 - DNA, 250 bp, synthetic construct
  misc_feature 1..250: note = SYNTHETIC PROMOTER
  source 1..250: mol_type = other DNA
tacagggacagcagagatccagtttggactagcccggtcgcactagttctagaacttcccggaagtagggtgggcaagtacttcccggaagttctagaggaaattttcggggactttccgggggttctctctagatattaaggtgacgcgtgtggcctcgaacaccgagcgaccctgcagcgacccgcttaaaagcggccgccatgggccgccatggcctcctccgaggacgtcatcaaggagttcatgc

SEQ ID NO: 24 - DNA, 250 bp, synthetic construct
  misc_feature 1..250: note = SYNTHETIC PROMOTER
  source 1..250: mol_type = other DNA
tacagggacagcagagatccagtttggactagcccggtcgcactagttctagaacttcccggaagtagggtgggcaagtacttccgggaaattctagagggagttctcggggactttccgggaattttctctagatattaaggtgacgcgtgtggcctcgaacaccgagcgaccctgcagcgacccgcttaaaagcggccgccatgggccgccatggcctcctccgaggacgtcatcaaggagttcatgc

SEQ ID NO: 25 - DNA, 250 bp, synthetic construct
  misc_feature 1..250: note = SYNTHETIC PROMOTER
  source 1..250: mol_type = other DNA
tacagggacagcagagatccagtttggactagcccggtcgcactagttctagaacttcccggaagtagggtgggcaagtatttcccggaagttctagaggaagttctcggggactttccggagattctctctagatattaaggtgacgcgtgtggcctcgaacaccgagcgaccctgcagcgacccgcttaaaagcggccgccatgggccgccatggcctcctccgaggacgtcatcaaggagttcatgc

SEQ ID NO: 26 - DNA, 250 bp, synthetic construct
  misc_feature 1..250: note = SYNTHETIC PROMOTER
  source 1..250: mol_type = other DNA
tacagggacagcagagatccagtttggactagcccggtcgcactagttctagaacttccgggaaatagggtgggcaagtacttccgggaaattctagaggggatttccggggactttccggaggttctctctagatattaaggtgacgcgtgtggcctcgaacaccgagcgaccctgcagcgacccgcttaaaagcggccgccatgggccgccatggcctcctccgaggacgtcatcaaggagttcatgc

SEQ ID NO: 27 - DNA, 250 bp, synthetic construct
  misc_feature 1..250: note = SYNTHETIC PROMOTER
  source 1..250: mol_type = other DNA
tacagggacagcagagatccagtttggactagcccggtcgcactagttctagaacttccgggaaatagggtgggcaagtacttccgggaagttctagaggaggttttcggggactttccggaggtttcctctagatattaaggtgacgcgtgtggcctcgaacaccgagcgaccctgcagcgacccgcttaaaagcggccgccatgggccgccatggcctcctccgaggacgtcatcaaggagttcatgc

SEQ ID NO: 28 - DNA, 250 bp, synthetic construct
  misc_feature 1..250: note = SYNTHETIC PROMOTER
  source 1..250: mol_type = other DNA
tacagggacagcagagatccagtttggactagcccggtcgcactagttctagaacttccgggaagtagggtgggcaagtatttcccggaagttctagagggggttttcggggactttccggaggtttcctctagatattaaggtgacgcgtgtggcctcgaacaccgagcgaccctgcagcgacccgcttaaaagcggccgccatgggccgccatggcctcctccgaggacgtcatcaaggagttcatgc

SEQ ID NO: 29 - DNA, 250 bp, synthetic construct
  misc_feature 1..250: note = SYNTHETIC PROMOTER
  source 1..250: mol_type = other DNA
tacagggacagcagagatccagtttggactagcccggtcgcactagttctagaacttccgggaagtagggtgggcaagtatttccgggaaattctagagggagttctcggggactttccggggattttctctagatattaaggtgacgcgtgtggcctcgaacaccgagcgaccctgcagcgacccgcttaaaagcggccgccatgggccgccatggcctcctccgaggacgtcatcaaggagttcatgc

SEQ ID NO: 30 - DNA, 250 bp, synthetic construct
  misc_feature 1..250: note = SYNTHETIC PROMOTER
  source 1..250: mol_type = other DNA
tacagggacagcagagatccagtttggactagcccggtcgcactagttctagaatttcccggaaatagggtgggcaagtacttccgggaaattctagagggggtttccggggactttccgggggttttctctagatattaaggtgacgcgtgtggcctcgaacaccgagcgaccctgcagcgacccgcttaaaagcggccgccatgggccgccatggcctcctccgaggacgtcatcaaggagttcatgc

SEQ ID NO: 31 - DNA, 250 bp, synthetic construct
  misc_feature 1..250: note = SYNTHETIC PROMOTER
  source 1..250: mol_type = other DNA
tacagggacagcagagatccagtttggactagcccggtcgcactagttctagaatttcccggaaatagggtgggcaagtatttcccggaaattctagagggggttttcggggactttccgggaattttctctagatattaaggtgacgcgtgtggcctcgaacaccgagcgaccctgcagcgacccgcttaaaagcggccgccatgggccgccatggcctcctccgaggacgtcatcaaggagttcatgc

SEQ ID NO: 32 - DNA, 250 bp, synthetic construct
  misc_feature 1..250: note = SYNTHETIC PROMOTER
  source 1..250: mol_type = other DNA
tacagggacagcagagatccagtttggactagcccggtcgcactagttctagaatttcccggaaatagggtgggcaagtatttccgggaaattctagaggaggttctcggggactttccgggagttttctctagatattaaggtgacgcgtgtggcctcgaacaccgagcgaccctgcagcgacccgcttaaaagcggccgccatgggccgccatggcctcctccgaggacgtcatcaaggagttcatgc

SEQ ID NO: 33 - DNA, 250 bp, synthetic construct
  misc_feature 1..250: note = SYNTHETIC PROMOTER
  source 1..250: mol_type = other DNA
tacagggacagcagagatccagtttggactagcccggtcgcactagttctagaatttcccggaaatagggtgggcaagtatttccgggaaattctagaggaggttttcggggactttccgggagtttcctctagatattaaggtgacgcgtgtggcctcgaacaccgagcgaccctgcagcgacccgcttaaaagcggccgccatgggccgccatggcctcctccgaggacgtcatcaaggagttcatgc

SEQ ID NO: 34 - DNA, 250 bp, synthetic construct
  misc_feature 1..250: note = SYNTHETIC PROMOTER
  source 1..250: mol_type = other DNA
tacagggacagcagagatccagtttggactagcccggtcgcactagttctagaatttcccggaaatagggtgggcaagtatttccgggaagttctagaggaagttttcggggactttccgggaattttctctagatattaaggtgacgcgtgtggcctcgaacaccgagcgaccctgcagcgacccgcttaaaagcggccgccatgggccgccatggcctcctccgaggacgtcatcaaggagttcatgc

SEQ ID NO: 35 - DNA, 250 bp, synthetic construct
  misc_feature 1..250: note = SYNTHETIC PROMOTER
  source 1..250: mol_type = other DNA
tacagggacagcagagatccagtttggactagcccggtcgcactagttctagaatttccgggaaatagggtgggcaagtatttcccggaagttctagaggagattctcggggactttccgggggttctctctagatattaaggtgacgcgtgtggcctcgaacaccgagcgaccctgcagcgacccgcttaaaagcggccgccatgggccgccatggcctcctccgaggacgtcatcaaggagttcatgc

SEQ ID NO: 36 - DNA, 250 bp, synthetic construct
  misc_feature 1..250: note = SYNTHETIC PROMOTER
  source 1..250: mol_type = other DNA
tacagggacagcagagatccagtttggactagcccggtcgcactagttctagaatttccgggaagtagggtgggcaagtacttccgggaaattctagagggggtttccggggactttccggagattctctctagatattaaggtgacgcgtgtggcctcgaacaccgagcgaccctgcagcgacccgcttaaaagcggccgccatgggccgccatggcctcctccgaggacgtcatcaaggagttcatgc

SEQ ID NO: 37 - DNA, 249 bp, synthetic construct
  misc_feature 1..249: note = SYNTHETIC PROMOTER
  source 1..249: mol_type = other DNA
tacagggacagcagagatccagtttggactagcccggtcgcactagttctagaatttccgggaaatagggtgggcaagtatttcccggaagttctagagggggttttcggggactttccggaaattttctctagatattaaggtgacgcgtgtggcctcgaacaccgagcgaccctgcagcgacccgcttaaaagcggccgccatgggccccatggcctcctccgaggacgtcatcaaggagttcatgc

SEQ ID NO: 38 - DNA, 249 bp, synthetic construct
  misc_feature 1..249: note = SYNTHETIC PROMOTER
  source 1..249: mol_type = other DNA
tacagggacagcagagatccagtttggactagcccggtcgcactagttctagaacttcccggaaatagggtgggcaagtatttcccggaagttctagaggaggttttcggggactttccgggattccctctagatattaaggtgacgcgtgtggcctcgaacaccgagcgaccctgcagcgacccgcttaaaagcggccgccatgggccgccatggcctcctccgaggacgtcatcaaggagttcatgc

SEQ ID NO: 39 - DNA, 243 bp, synthetic construct
  misc_feature 1..243: note = SYNTHETIC PROMOTER
  source 1..243: mol_type = other DNA
tacagggacagcagagatccagtttggactagcccggtcgcactagttctagttccgggaagtgggtgggcaatatttcccggaagtttagaggaagttttcggggacttccggaaattccctctagatattaaggtgacgcgtgtggcctcgaacaccgagcgaccctgcagcgacccgcttaaaagcggccgccatgggccgccatggcctcctccgaggacgtcatcaaggagttcatgc

SEQ ID NO: 40 - DNA, 200 bp, synthetic construct
  misc_feature 1..200: note = SYNTHETIC PROMOTER
  source 1..200: mol_type = other DNA
tacagggacagcagagatccagtttggactagcccggtcgcactagttctagaacttctcggaaatagggtgggcaagtactgtggcctcgaacaccgagcgaccctgcagcgacccgcttaaaagcggccgccatgggccgccatggcctcctccgaggacgtcatcaaggagttcatgcagaccaagtctctgctacc

SEQ ID NO: 41 - DNA, 250 bp, synthetic construct
  misc_feature 1..250: note = SYNTHETIC PROMOTER
  source 1..250: mol_type = other DNA
tacagggacagcagagatccagtttggactagcccggtcgcactagttctagaayttccsggaartagggtgggcaagtayttccsggaarttctagaggrrrttyycggggactttccggrrrttyyctctagatattaaggtgacgcgtgtggcctcgaacaccgagcgaccctgcagcgacccgcttaaaagcggccgccatgggccgccatggcctcctccgaggacgtcatcaaggagttcatgc

SEQ ID NO: 42 - DNA, 50 bp, synthetic construct
  source 1..50: mol_type = other DNA
acgtggctggagtcacagtcctcttacgtggctggagtcacagtcctctt

SEQ ID NO: 43 - DNA, 50 bp, synthetic construct
  source 1..50: mol_type = other DNA
rcgtgsctggagtmacagtcctcttrcgtgsctggagtmacagtcctctt

SEQ ID NO: 44 - DNA, 39 bp, synthetic construct
  source 1..39: mol_type = other DNA
acttccsggaartagggtgggcaagtacttccsggaart

SEQ ID NO: 45 - DNA, 30 bp, synthetic construct
  source 1..30: mol_type = other DNA
gggggtttycggggactttccggrrrtttt

SEQ ID NO: 46 - DNA, 255 bp, synthetic construct
  source 1..255: mol_type = other DNA
acgtggctggagtcacagtcctcttacgtggctggagtcacagtcctcttactagttctagaacttcccggaagtagggtgggcaagtacttcccggaagttctagaggaaattttcggggactttccgggggttctctctagatattaaggtgacgcgtgtggcctcgaacaccgagcgaccctgcagcgacccgcttaaaagcggccgccatgggccgccatggcctcctccgaggacgtcatcaaggagttc

SEQ ID NO: 47 - DNA, 255 bp, synthetic construct
  source 1..255: mol_type = other DNA
aagaggactgtgactccagccacgtaagaggactgtgactccagccacgtactagttctagaacttcccggaagtagggtgggcaagtacttcccggaagttctagaggaaattttcggggactttccgggggttctctctagatattaaggtgacgcgtgtggcctcgaacaccgagcgaccctgcagcgacccgcttaaaagcggccgccatgggccgccatggcctcctccgaggacgtcatcaaggagttc